European Patent Application EP 4 485 298 A1, published January 1, 2025. Title: CONDITION OPTIMIZATION DEVICE, CONDITION OPTIMIZATION METHOD, AND PROGRAM. Applicant: 日東電工株式会社. Application WO PCT/JP2023/006148, filed February 21, 2023. The sequence listing filed with the application follows.

SEQUENCE LISTING (1 sequence)

SEQ ID NO: 1 - DNA, 24 bp, synthetic construct
  source 1..24: mol_type = other DNA; note = all oxidized
tcgacgtattgacgtattgacgta